European Patent Application EP 4 116 325 A1, published January 11, 2023. Title: METHODS OF TREATING RHEUMATOID ARTHRITIS USING IL-17 BINDING MOLECULES. Applicant: Novartis AG Richards, Hanno Mpofu, Shephard Thangavelu, Karthinathan. Application Herewith. The sequence listing filed with the application follows.

SEQUENCE LISTING (17 sequences)

SEQ ID NO: 1 - protein, 5 aa, artificial
  CDR1 = hypervariable region 1 of heavy chain of AIN457
NYWMN

SEQ ID NO: 2 - protein, 17 aa, ARTIFICIAL
  CDR2 = hypervariable region 2 of heavy chain of AIN457
AINQDGSEKYYVGSVKG

SEQ ID NO: 3 - protein, 18 aa, ARTIFICIAL
  CDR3 = hypervariable region 3 of heavy chain of AIN457
DYYDILTDYYIHYWYFDL

SEQ ID NO: 4 - protein, 12 aa, ARTIFICIAL
  CDR1' = hypervariable region 1 of light chain of AIN457
RASQSVSSSYLA

SEQ ID NO: 5 - protein, 7 aa, ARTIFICIAL
  CDR2' = hypervariable region 2 of light chain AIN457
GASSRAT

SEQ ID NO: 6 - protein, 9 aa, ARTIFICIAL
  CDR3' = hypervariable region 3 of light chain AIN457
QQYGSSPCT

SEQ ID NO: 7 - DNA, 381 bp, HOMO SAPIENS
  CDS (1)..(381)
gaggtgcagttggtggagtctgggggaggcttggtccagcctggggggtccctgagactctcctgtgcagcctctggattcacctttagtaactattggatgaactgggtccgccaggctccagggaaagggctggagtgggtggccgccataaaccaagatggaagtgagaaatactatgtgggctctgtgaagggccgattcaccatctccagagacaacgccaagaactcactgtatctgcaaatgaacagcctgagagtcgaggacacggctgtgtattactgtgtgagggactattacgatattttgaccgattattacatccactattggtacttcgatctctggggccgtggcaccctggtcactgtctcctca

SEQ ID NO: 8 - protein, 127 aa, HOMO SAPIENS [sequence omitted]

SEQ ID NO: 9 - DNA, 327 bp, HOMO SAPIENS
  CDS (1)..(327)
gaaattgtgttgacgcagtctccaggcaccctgtctttgtctccaggggaaagagccaccctctcctgcagggccagtcagagtgttagcagcagctacttagcctggtaccagcagaaacctggccaggctcccaggctcctcatctatggtgcatccagcagggccactggcatcccagacaggttcagtggcagtgggtctgggacagacttcactctcaccatcagcagactggagcctgaagattttgcagtgtattactgtcagcagtatggtagctcaccgtgcaccttcggccaagggacacgactggagattaaacga

SEQ ID NO: 10 - protein, 109 aa, HOMO SAPIENS
EIVLTQSPGTLSLSPGERATLSCRASQSVSSSYLAWYQQKPGQAPRLLIYGASSRATGIPDRFSGSGSGTDFTLTISRLEPEDFAVYYCQQYGSSPCTFGQGTRLEIKR

SEQ ID NO: 11 - protein, 10 aa, artificial
  CDR1-x = hypervariable domain x of heavy chain of AIN457
GFTFSNYWMN

SEQ ID NO: 12 - protein, 11 aa, artificial
  CDR2-x = hypervariable domain of heavy chain x of AIN457
AINQDGSEKYY

SEQ ID NO: 13 - protein, 23 aa, ARTIFICIAL
  CDR3-x = hypervariable domain x of heavy chain AIN457
CVRDYYDILTDYYIHYWYFDLWG

SEQ ID NO: 14 - DNA, 711 bp, homo sapiens
  CDS (1)..(708)
accatggaaaccccagcggagcttctcttcctcctgctactctggctcccagataccaccggagaaattgtgttgacgcagtctccaggcaccctgtctttgtctccaggggaaagagccaccctctcctgcagggccagtcagagtgttagcagcagctacttagcctggtaccagcagaaacctggccaggctcccaggctcctcatctatggtgcatccagcagggccactggcatcccagacaggttcagtggcagtgggtctgggacagacttcactctcaccatcagcagactggagcctgaagattttgcagtgtattactgtcagcagtatggtagctcaccgtgcaccttcggccaagggacacgactggagattaaacgaactgtggctgcaccatctgtcttcatcttcccgccatctgatgagcagttgaaatctggaactgcctctgttgtgtgcctgctgaataacttctatcccagagaggccaaagtacagtggaaggtggataacgccctccaatcgggtaactcccaggagagtgtcacagagcaggacagcaaggacagcacctacagcctcagcagcaccctgacgctgagcaaagcagactacgagaaacacaaagtctacgcctgcgaagtcacccatcagggcctgagctcgcccgtcacaaagagcttcaacaggggagagtgttag

SEQ ID NO: 15 - protein, 236 aa, homo sapiens
TMETPAELLFLLLLWLPDTTGEIVLTQSPGTLSLSPGERATLSCRASQSVSSSYLAWYQQKPGQAPRLLIYGASSRATGIPDRFSGSGSGTDFTLTISRLEPEDFAVYYCQQYGSSPCTFGQGTRLEIKRTVAAPSVFIFPPSDEQLKSGTASVVCLLNNFYPREAKVQWKVDNALQSGNSQESVTEQDSKDSTYSLSSTLTLSKADYEKHKVYACEVTHQGLSSPVTKSFNRGEC

SEQ ID NO: 16 - DNA, 783 bp, homo sapiens
  CDS (1)..(780)
accatggaattggggctgagctgggttttccttgttgctattttagaaggtgtccactgtgaggtgcagttggtggagtctgggggaggcttggtccagcctggggggtccctgagactctcctgtgcagcctctggattcacctttagtaactattggatgaactgggtccgccaggctccagggaaagggctggagtgggtggccgccataaaccaagatggaagtgagaaatactatgtgggctctgtgaagggccgattcaccatctccagagacaacgccaagaactcactgtatctgcaaatgaacagcctgagagtcgaggacacggctgtgtattactgtgtgagggactattacgatattttgaccgattattacatccactattggtacttcgatctctggggccgtggcaccctggtcactgtctcctcagcctccaccaagggcccatcggtcttccccctggcaccctcctccaagagcacctctgggggcacagcggccctgggctgcctggtcaaggactacttccccgaaccggtgacggtgtcgtggaactcaggcgccctgaccagcggcgtgcacaccttcccggctgtcctacagtcctcaggactctactccctcagcagcgtggtgaccgtgccctccagcagcttgggcacccagacctacatctgcaacgtgaatcacaagcccagcaacaccaaggtggacaagagagttgagcccaaatcttgtgacaaaactcacacatgcccaccgtgcccataa

SEQ ID NO: 17 - protein, 260 aa, homo sapiens
TMELGLSWVFLVAILEGVHCEVQLVESGGGLVQPGGSLRLSCAASGFTFSNYWMNWVRQAPGKGLEWVAAINQDGSEKYYVGSVKGRFTISRDNAKNSLYLQMNSLRVEDTAVYYCVRDYYDILTDYYIHYWYFDLWGRGTLVTVSSASTKGPSVFPLAPSSKSTSGGTAALGCLVKDYFPEPVTVSWNSGALTSGVHTFPAVLQSSGLYSLSSVVTVPSSSLGTQTYICNVNHKPSNTKVDKRVEPKSCDKTHTCPPCP